European Patent Application EP 4 119 153 A1, published January 18, 2023. Title: CD47 TARGETED THERAPIES FOR THE TREATMENT OF INFECTIOUS DISEASE. Applicant: The Board of Trustees of the Leland Stanford Junior University. The sequence listing filed with the application follows.

SEQUENCE LISTING (3 sequences)

SEQ ID NO: 1 - protein, 124 aa, Homo sapiens
QLLFNKTKSVEFTFCNDTVVIPCFVTNMEAQNTTEVYVKWKFKGRDIYTFDGALNKSTVPTDFSSAKIEVSQLLKGDASLKMDKSDAVSHTGNYTCEVTELTREGETIIELKYRVVSWFSPNEN

SEQ ID NO: 2 - protein, 18 aa, synthetic construct
  REGION 1..18: note = Sythetic polypeptide sequence
MWPLVAALLLGSACCGSA

SEQ ID NO: 3 - protein, 142 aa, Homo sapiens
MWPLVAALLLGSACCGSAQLLFNKTKSVEFTFCNDTVVIPCFVTNMEAQNTTEVYVKWKFKGRDIYTFDGALNKSTVPTDFSSAKIEVSQLLKGDASLKMDKSDAVSHTGNYTCEVTELTREGETIIELKYRVVSWFSPNEN